European Patent Application EP 4 763 866 A1, published June 24, 2026. Title: ANTI-PD-1-ANTI-VEGFA BISPECIFIC ANTIBODY, PHARMACEUTICAL COMPOSITION AND USE THEREOF. Applicant: AKESO BIOPHARMA, INC. Application EP. The sequence listing filed with the application follows.

SEQUENCE LISTING (42 sequences)

SEQ ID NO: 1 - protein, 123 aa, synthetic construct [sequence omitted]

SEQ ID NO: 2 - DNA, 369 bp, synthetic construct
  misc_feature 1..369: note = nucleic acid encoding Bevacizumab-Hv
  source 1..369: mol_type = other DNA
gaggtgcagctggtcgagtccgggggggggctggtgcagccaggcgggtctctgaggctgagttgcgccgcttcagggtacaccttcacaaactatggaatgaattgggtgcgccaggcaccaggaaagggactggagtgggtcggctggatcaacacttacaccggggaacctacctatgcagccgactttaagcggcggttcaccttcagcctggatacaagcaaatccactgcctacctgcagatgaacagcctgcgagctgaggacaccgcagtctactattgtgctaaatatccccactactatgggagcagccattggtattttgacgtgtgggggcaggggactctggtgacagtgagcagc

SEQ ID NO: 3 - protein, 107 aa, synthetic construct [sequence omitted]

SEQ ID NO: 4 - DNA, 321 bp, synthetic construct
  misc_feature 1..321: note = nucleic acid encoding Bevacizumab-Lv
  source 1..321: mol_type = other DNA
gatattcagatgactcagagcccctcctccctgtccgcctctgtgggcgacagggtcaccatcacatgcagtgcttcacaggatatttccaactacctgaattggtatcagcagaagccaggaaaagcacccaaggtgctgatctacttcactagctccctgcactcaggagtgccaagccggttcagcggatccggatctggaaccgactttactctgaccatttctagtctgcagcctgaggatttcgctacatactattgccagcagtattctaccgtgccatggacatttggccaggggactaaagtcgagatcaag

SEQ ID NO: 5 - protein, 118 aa, synthetic construct
  REGION 1..118: note = VH of 14C12
EVKLVESGGGLVKPGGSLKLSCAASGFAFSSYDMSWVRQTPEKRLEWVATISGGGRYTYYPDSVKGRFTISRDNARNTLYLQMSSLRSEDTALYYCANRYGEAWFAYWGQGTLVTVSA

SEQ ID NO: 6 - DNA, 354 bp, synthetic construct
  misc_feature 1..354: note = nucleic acid encoding VH of 14C12
  source 1..354: mol_type = other DNA
gaggtcaaactggtggagagcggcggcgggctggtgaagcccggcgggtcactgaaactgagctgcgccgcttccggcttcgcctttagctcctacgacatgtcatgggtgaggcagacccctgagaagcgcctggaatgggtcgctactatcagcggaggcgggcgatacacctactatcctgactctgtcaaagggagattcacaattagtcgggataacgccagaaatactctgtatctgcagatgtctagtctgcggtccgaggatacagctctgtactattgtgcaaaccggtacggcgaagcatggtttgcctattggggacagggcaccctggtgacagtctctgcc

SEQ ID NO: 7 - protein, 107 aa, synthetic construct
  REGION 1..107: note = VL of 14C12
DIKMTQSPSSMYASLGERVTFTCKASQDINTYLSWFQQKPGKSPKTLIYRANRLVDGVPSRFSGSGSGQDYSLTISSLEYEDMGIYYCLQYDEFPLTFGAGTKLELK

SEQ ID NO: 8 - DNA, 321 bp, synthetic construct
  misc_feature 1..321: note = nucleic acid encoding VL of 14C12
  source 1..321: mol_type = other DNA
gacattaagatgacacagtccccttcctcaatgtacgctagcctgggcgagcgagtgaccttcacatgcaaagcatcccaggacatcaacacatacctgtcttggtttcagcagaagccaggcaaaagccccaagaccctgatctaccgggccaatagactggtggacggggtccccagcagattctccggatctggcagtgggcaggattactccctgaccatcagctccctggagtatgaagacatgggcatctactattgcctgcagtatgatgagttccctctgacctttggagcaggcacaaaactggaactgaag

SEQ ID NO: 9 - protein, 118 aa, synthetic construct
  REGION 1..118: note = VH of 14C12H1L1
EVQLVESGGGLVQPGGSLRLSCAASGFAFSSYDMSWVRQAPGKGLDWVATISGGGRYTYYPDSVKGRFTISRDNSKNNLYLQMNSLRAEDTALYYCANRYGEAWFAYWGQGTLVTVSS

SEQ ID NO: 10 - DNA, 354 bp, synthetic construct
  misc_feature 1..354: note = nucleic acid encoding VH of 14C12H1L1
  source 1..354: mol_type = other DNA
gaagtgcagctggtcgagtctgggggagggctggtgcagcccggcgggtcactgcgactgagctgcgcagcttccggattcgcctttagctcctacgacatgtcctgggtgcgacaggcaccaggaaagggactggattgggtcgctactatctcaggaggcgggagatacacctactatcctgacagcgtcaagggccggttcacaatctctagagataacagtaagaacaatctgtatctgcagatgaacagcctgagggctgaggacaccgcactgtactattgtgccaaccgctacggggaagcatggtttgcctattgggggcagggaaccctggtgacagtctctagt

SEQ ID NO: 11 - protein, 107 aa, synthetic construct
  REGION 1..107: note = VL of 14C12H1L1
DIQMTQSPSSMSASVGDRVTFTCRASQDINTYLSWFQQKPGKSPKTLIYRANRLVSGVPSRFSGSGSGQDYTLTISSLQPEDMATYYCLQYDEFPLTFGAGTKLELK

SEQ ID NO: 12 - DNA, 321 bp, synthetic construct
  misc_feature 1..321: note = nucleic acid encoding VL of 14C12H1L1
  source 1..321: mol_type = other DNA
gacattcagatgactcagagcccctcctccatgtccgcctctgtgggcgacagggtcaccttcacatgccgcgctagtcaggatatcaacacctacctgagctggtttcagcagaagccagggaaaagccccaagacactgatctaccgggctaatagactggtgtctggagtcccaagtcggttcagtggctcagggagcggacaggactacactctgaccatcagctccctgcagcctgaggacatggcaacctactattgcctgcagtatgatgagttcccactgacctttggcgccgggacaaaactggagctgaag

SEQ ID NO: 13 - protein, 448 aa, synthetic construct
  REGION 1..448: note = heavy chain of 14C12H1L1
EVQLVESGGGLVQPGGSLRLSCAASGFAFSSYDMSWVRQAPGKGLDWVATISGGGRYTYYPDSVKGRFTISRDNSKNNLYLQMNSLRAEDTALYYCANRYGEAWFAYWGQGTLVTVSSASTKGPSVFPLAPSSKSTSGGTAALGCLVKDYFPEPVTVSWNSGALTSGVHTFPAVLQSSGLYSLSSVVTVPSSSLGTQTYICNVNHKPSNTKVDKKVEPKSCDKTHTCPPCPAPELLGGPSVFLFPPKPKDTLMISRTPEVTCVVVDVSHEDPEVKFNWYVDGVEVHNAKTKPREEQYNSTYRVVSVLTVLHQDWLNGKEYKCKVSNKALPAPIEKTISKAKGQPREPQVYTLPPSRDELTKNQVSLTCLVKGFYPSDIAVEWESNGQPENNYKTTPPVLDSDGSFFLYSKLTVDKSRWQQGNVFSCSVMHEALHNHYTQKSLSLSPGK

SEQ ID NO: 14 - DNA, 1344 bp, synthetic construct
  misc_feature 1..1344: note = nucleic acid encoding heavy chain of 14C12H1L1
  source 1..1344: mol_type = other DNA
gaagtgcagctggtcgagtctgggggagggctggtgcagcccggcgggtcactgcgactgagctgcgcagcttccggattcgcctttagctcctacgacatgtcctgggtgcgacaggcaccaggaaagggactggattgggtcgctactatctcaggaggcgggagatacacctactatcctgacagcgtcaagggccggttcacaatctctagagataacagtaagaacaatctgtatctgcagatgaacagcctgagggctgaggacaccgcactgtactattgtgccaaccgctacggggaagcatggtttgcctattgggggcagggaaccctggtgacagtctctagtgccagcaccaaaggacctagcgtgtttcctctcgccccctcctccaaaagcaccagcggaggaaccgctgctctcggatgtctggtgaaggactacttccctgaacccgtcaccgtgagctggaatagcggcgctctgacaagcggagtccatacattccctgctgtgctgcaaagcagcggactctattccctgtccagcgtcgtcacagtgcccagcagcagcctgggcacccagacctacatctgtaacgtcaaccacaagccctccaacaccaaggtggacaagaaagtggagcccaaatcctgcgacaagacacacacctgtcccccctgtcctgctcccgaactcctcggaggccctagcgtcttcctctttcctcccaaacccaaggacaccctcatgatcagcagaacccctgaagtcacctgtgtcgtcgtggatgtcagccatgaggaccccgaggtgaaattcaactggtatgtcgatggcgtcgaggtgcacaacgccaaaaccaagcccagggaggaacagtacaactccacctacagggtggtgtccgtgctgacagtcctccaccaggactggctgaacggcaaggagtacaagtgcaaggtgtccaacaaggctctccctgcccccattgagaagaccatcagcaaggccaaaggccaacccagggagccccaggtctatacactgcctccctccagggacgaactcaccaagaaccaggtgtccctgacctgcctggtcaagggcttttatcccagcgacatcgccgtcgagtgggagtccaacggacagcccgagaataactacaagaccacccctcctgtcctcgactccgacggctccttcttcctgtacagcaagctgaccgtggacaaaagcaggtggcagcagggaaacgtgttctcctgcagcgtgatgcacgaagccctccacaaccactacacccagaaaagcctgtccctgagccccggcaaa

SEQ ID NO: 15 - protein, 214 aa, synthetic construct
  REGION 1..214: note = light chain of 14C12H1L1
DIQMTQSPSSMSASVGDRVTFTCRASQDINTYLSWFQQKPGKSPKTLIYRANRLVSGVPSRFSGSGSGQDYTLTISSLQPEDMATYYCLQYDEFPLTFGAGTKLELKRTVAAPSVFIFPPSDEQLKSGTASVVCLLNNFYPREAKVQWKVDNALQSGNSQESVTEQDSKDSTYSLSSTLTLSKADYEKHKVYACEVTHQGLSSPVTKSFNRGEC

SEQ ID NO: 16 - DNA, 642 bp, synthetic construct
  misc_feature 1..642: note = lnucleic acid encoding ight chain of 14C12H1L1
  source 1..642: mol_type = other DNA
gacattcagatgactcagagcccctcctccatgtccgcctctgtgggcgacagggtcaccttcacatgccgcgctagtcaggatatcaacacctacctgagctggtttcagcagaagccagggaaaagccccaagacactgatctaccgggctaatagactggtgtctggagtcccaagtcggttcagtggctcagggagcggacaggactacactctgaccatcagctccctgcagcctgaggacatggcaacctactattgcctgcagtatgatgagttcccactgacctttggcgccgggacaaaactggagctgaagcgaactgtggccgctccctccgtcttcatttttcccccttctgacgaacagctgaaatcaggcacagccagcgtggtctgtctgctgaacaatttctaccctagagaggcaaaagtgcagtggaaggtcgataacgccctgcagtccggcaacagccaggagagtgtgactgaacaggactcaaaagatagcacctattccctgtctagtacactgactctgtccaaggctgattacgagaagcacaaagtgtatgcatgcgaagtgacacatcagggactgtcaagccccgtgactaagtcttttaaccggggcgaatgt

SEQ ID NO: 17 - protein, 108 aa, synthetic construct
  REGION 1..108: note = light chain of 14C12H1L1(M)1
DIQMTQSPSSMSASVGDRVTFTCRASQDINTYLSWFQQKPGKSPKTLIYRANRLVSGVPSRFSGSGSGQDYTLTISSLQPEDMATYYCLQYDEFPLTFGAGTKLELKR

SEQ ID NO: 18 - protein, 20 aa, synthetic construct
  REGION 1..20: note = Linker 1
GGGGSGGGGSGGGGSGGGGS

SEQ ID NO: 19 - protein, 15 aa, synthetic construct
  REGION 1..15: note = linker 2
GGGGSGGGGSGGGGS

SEQ ID NO: 20 - protein, 453 aa, synthetic construct
  REGION 1..453: note = Bevacizumab-G4H
EVQLVESGGGLVQPGGSLRLSCAASGYTFTNYGMNWVRQAPGKGLEWVGWINTYTGEPTYAADFKRRFTFSLDTSKSTAYLQMNSLRAEDTAVYYCAKYPHYYGSSHWYFDVWGQGTLVTVSSASTKGPSVFPLAPSSKSTSGGTAALGCLVKDYFPEPVTVSWNSGALTSGVHTFPAVLQSSGLYSLSSVVTVPSSSLGTQTYICNVNHKPSNTKVDKKVEPKSCDKTHTCPPCPAPELLGGPSVFLFPPKPKDTLMISRTPEVTCVVVDVSHEDPEVKFNWYVDGVEVHNAKTKPREEQYNSTYRVVSVLTVLHQDWLNGKEYKCKVSNKALPAPIEKTISKAKGQPREPQVYTLPPSRDELTKNQVSLTCLVKGFYPSDIAVEWESNGQPENNYKTTPPVLDSDGSFFLYSKLTVDKSRWQQGNVFSCSVMHEALHNHYTQKSLSLSPGK

SEQ ID NO: 21 - DNA, 1359 bp, synthetic construct
  misc_feature 1..1359: note = nucleic acid encoding Bevacizumab-G4H
  source 1..1359: mol_type = other DNA
gaggtgcagctggtcgagtccgggggggggctggtgcagccaggcgggtctctgaggctgagttgcgccgcttcagggtacaccttcacaaactatggaatgaattgggtgcgccaggcaccaggaaagggactggagtgggtcggctggatcaacacttacaccggggaacctacctatgcagccgactttaagcggcggttcaccttcagcctggatacaagcaaatccactgcctacctgcagatgaacagcctgcgagctgaggacaccgcagtctactattgtgctaaatatccccactactatgggagcagccattggtattttgacgtgtgggggcaggggactctggtgacagtgagcagcgcaagcaccaaagggcccagcgtgtttcctctcgccccctcctccaaaagcaccagcggaggaaccgctgctctcggatgtctggtgaaggactacttccctgaacccgtcaccgtgagctggaatagcggcgctctgacaagcggagtccatacattccctgctgtgctgcaaagcagcggactctattccctgtccagcgtcgtcacagtgcccagcagcagcctgggcacccagacctacatctgtaacgtcaaccacaagccctccaacaccaaggtggacaagaaagtggagcccaaatcctgcgacaagacacacacctgtcccccctgtcctgctcccgaactcctcggaggccctagcgtcttcctctttcctcccaaacccaaggacaccctcatgatcagcagaacccctgaagtcacctgtgtcgtcgtggatgtcagccatgaggaccccgaggtgaaattcaactggtatgtcgatggcgtcgaggtgcacaacgccaaaaccaagcccagggaggaacagtacaactccacctacagggtggtgtccgtgctgacagtcctccaccaggactggctgaacggcaaggagtacaagtgcaaggtgtccaacaaggctctccctgcccccattgagaagaccatcagcaaggccaaaggccaacccagggagccccaggtctatacactgcctccctccagggacgaactcaccaagaaccaggtgtccctgacctgcctggtcaagggcttttatcccagcgacatcgccgtcgagtgggagtccaacggacagcccgagaataactacaagaccacccctcctgtcctcgactccgacggctccttcttcctgtacagcaaactgaccgtcgataaatctaggtggcagcagggcaacgtgttctcttgttccgtgatgcatgaagcactgcacaaccattatacccagaagtctctgagcctgtcccccggcaag

SEQ ID NO: 22 - protein, 450 aa, synthetic construct
  REGION 1..450: note = heavy chain of VP101(hG4WT)
EVQLVESGGGLVQPGGSLRLSCAASGYTFTNYGMNWVRQAPGKGLEWVGWINTYTGEPTYAADFKRRFTFSLDTSKSTAYLQMNSLRAEDTAVYYCAKYPHYYGSSHWYFDVWGQGTLVTVSSASTKGPSVFPLAPCSRSTSESTAALGCLVKDYFPEPVTVSWNSGALTSGVHTFPAVLQSSGLYSLSSVVTVPSSSLGTKTYTCNVDHKPSNTKVDKRVESKYGPPCPPCPAPEFLGGPSVFLFPPKPKDTLMISRTPEVTCVVVDVSQEDPEVQFNWYVDGVEVHNAKTKPREEQFNSTYRVVSVLTVLHQDWLNGKEYKCKVSNKGLPSSIEKTISKAKGQPREPQVYTLPPSQEEMTKNQVSLTCLVKGFYPSDIAVEWESNGQPENNYKTTPPVLDSDGSFFLYSRLTVDKSRWQEGNVFSCSVMHEALHNHYTQKSLSLSLGK

SEQ ID NO: 23 - DNA, 1350 bp, synthetic construct
  misc_feature 1..1350: note = nucleic acid encoding heavy chain of VP101(hG4WT)
  source 1..1350: mol_type = other DNA
gaggtgcagctggtcgagtccgggggggggctggtgcagccaggcgggtctctgaggctgagttgcgccgcttcagggtacaccttcacaaactatggaatgaattgggtgcgccaggcaccaggaaagggactggagtgggtcggctggatcaacacttacaccggggaacctacctatgcagccgactttaagcggcggttcaccttcagcctggatacaagcaaatccactgcctacctgcagatgaacagcctgcgagctgaggacaccgcagtctactattgtgctaaatatccccactactatgggagcagccattggtattttgacgtgtgggggcaggggactctggtgacagtgagcagcgcaagcaccaaagggccctcggtcttccccctggcgccctgctccaggagcacctccgagagcacagccgccctgggctgcctggtcaaggactacttccccgaaccggtgacggtgtcgtggaactcaggcgccctgaccagcggcgtgcacaccttcccggctgtcctacagtcctcaggactctactccctcagcagcgtggtgaccgtgccctccagcagcttgggcacgaagacctacacctgcaacgtagatcacaagcccagcaacaccaaggtggacaagagagttgagtccaaatatggtcccccatgcccaccatgcccagcacctgagttcctggggggaccatcagtcttcctgttccccccaaaacccaaggacactctcatgatctcccggacccctgaggtcacgtgcgtggtggtggacgtgagccaggaagaccccgaggtccagttcaactggtacgtggatggcgtggaggtgcataatgccaagacaaagccgcgggaggagcagttcaacagcacgtaccgtgtggtcagcgtcctcaccgtcctgcaccaggactggctgaacggcaaggagtacaagtgcaaggtctccaacaaaggcctcccgtcctccatcgagaaaaccatctccaaagccaaagggcagccccgagagccacaggtgtacaccctgcccccatcccaggaggagatgaccaagaaccaggtcagcctgacctgcctggtcaaaggcttctaccccagcgacatcgccgtggagtgggagagcaatgggcagccggagaacaactacaagaccacgcctcccgtgctggactccgacggctccttcttcctctacagcaggctaaccgtggacaagagcaggtggcaggaggggaatgtcttctcatgctccgtgatgcatgaggctctgcacaaccactacacacagaagtctctgagcctgtccctcggcaag

SEQ ID NO: 24 - protein, 453 aa, synthetic construct
  REGION 1..453: note = Immunoglobulin heavy chain of VP101(hG1DM)
EVQLVESGGGLVQPGGSLRLSCAASGYTFTNYGMNWVRQAPGKGLEWVGWINTYTGEPTYAADFKRRFTFSLDTSKSTAYLQMNSLRAEDTAVYYCAKYPHYYGSSHWYFDVWGQGTLVTVSSASTKGPSVFPLAPSSKSTSGGTAALGCLVKDYFPEPVTVSWNSGALTSGVHTFPAVLQSSGLYSLSSVVTVPSSSLGTQTYICNVNHKPSNTKVDKKVEPKSCDKTHTCPPCPAPEAAGGPSVFLFPPKPKDTLMISRTPEVTCVVVDVSHEDPEVKFNWYVDGVEVHNAKTKPREEQYNSTYRVVSVLTVLHQDWLNGKEYKCKVSNKALPAPIEKTISKAKGQPREPQVYTLPPSRDELTKNQVSLTCLVKGFYPSDIAVEWESNGQPENNYKTTPPVLDSDGSFFLYSKLTVDKSRWQQGNVFSCSVMHEALHNHYTQKSLSLSPGK

SEQ ID NO: 25 - DNA, 1359 bp, synthetic construct
  misc_feature 1..1359: note = nucleic acid encoding Immunoglobulin heavy chain of VP101(hG1DM)
  source 1..1359: mol_type = other DNA
gaggtgcagctggtcgagtccgggggggggctggtgcagccaggcgggtctctgaggctgagttgcgccgcttcagggtacaccttcacaaactatggaatgaattgggtgcgccaggcaccaggaaagggactggagtgggtcggctggatcaacacttacaccggggaacctacctatgcagccgactttaagcggcggttcaccttcagcctggatacaagcaaatccactgcctacctgcagatgaacagcctgcgagctgaggacaccgcagtctactattgtgctaaatatccccactactatgggagcagccattggtattttgacgtgtgggggcaggggactctggtgacagtgagcagcgcaagcaccaaagggcccagcgtgtttcctctcgccccctcctccaaaagcaccagcggaggaaccgctgctctcggatgtctggtgaaggactacttccctgaacccgtcaccgtgagctggaatagcggcgctctgacaagcggagtccatacattccctgctgtgctgcaaagcagcggactctattccctgtccagcgtcgtcacagtgcccagcagcagcctgggcacccagacctacatctgtaacgtcaaccacaagccctccaacaccaaggtggacaagaaagtggagcccaaatcctgcgacaagacacacacctgtcccccctgtcctgctcccgaagctgctggaggccctagcgtcttcctctttcctcccaaacccaaggacaccctcatgatcagcagaacccctgaagtcacctgtgtcgtcgtggatgtcagccatgaggaccccgaggtgaaattcaactggtatgtcgatggcgtcgaggtgcacaacgccaaaaccaagcccagggaggaacagtacaactccacctacagggtggtgtccgtgctgacagtcctccaccaggactggctgaacggcaaggagtacaagtgcaaggtgtccaacaaggctctccctgcccccattgagaagaccatcagcaaggccaaaggccaacccagggagccccaggtctatacactgcctccctccagggacgaactcaccaagaaccaggtgtccctgacctgcctggtcaagggcttttatcccagcgacatcgccgtcgagtgggagtccaacggacagcccgagaataactacaagaccacccctcctgtcctcgactccgacggctccttcttcctgtacagcaaactgaccgtcgataaatctaggtggcagcagggcaacgtgttctcttgttccgtgatgcatgaagcactgcacaaccattatacccagaagtctctgagcctgtcccccggcaag

SEQ ID NO: 26 - protein, 214 aa, synthetic construct
  REGION 1..214: note = Immunoglobulin light chain of VP101(hG1DM)
DIQMTQSPSSLSASVGDRVTITCSASQDISNYLNWYQQKPGKAPKVLIYFTSSLHSGVPSRFSGSGSGTDFTLTISSLQPEDFATYYCQQYSTVPWTFGQGTKVEIKRTVAAPSVFIFPPSDEQLKSGTASVVCLLNNFYPREAKVQWKVDNALQSGNSQESVTEQDSKDSTYSLSSTLTLSKADYEKHKVYACEVTHQGLSSPVTKSFNRGEC

SEQ ID NO: 27 - DNA, 642 bp, synthetic construct
  misc_feature 1..642: note = nucleic acid encoding Immunoglobulin light chain of VP101(hG1DM)
  source 1..642: mol_type = other DNA
gatattcagatgactcagagcccctcctccctgtccgcctctgtgggcgacagggtcaccatcacatgcagtgcttcacaggatatttccaactacctgaattggtatcagcagaagccaggaaaagcacccaaggtgctgatctacttcactagctccctgcactcaggagtgccaagccggttcagcggatccggatctggaaccgactttactctgaccatttctagtctgcagcctgaggatttcgctacatactattgccagcagtattctaccgtgccatggacatttggccaggggactaaagtcgagatcaagcggaccgtggccgctcccagtgtcttcatttttccccctagcgacgaacagctgaaatccgggacagcctctgtggtctgtctgctgaacaacttctaccctagagaggcaaaagtgcagtggaaggtcgataacgccctgcagagtggcaattcacaggagagcgtgacagaacaggactccaaagattctacttatagtctgtcaagcacactgactctgagcaaggctgactacgaaaagcataaagtgtatgcatgtgaggtcacccaccaggggctgagcagtccagtcaccaagtcattcaacagaggcgagtgc

SEQ ID NO: 28 - protein, 8 aa, synthetic construct
  REGION 1..8: note = HCDR1
GYTFTNYG

SEQ ID NO: 29 - protein, 8 aa, synthetic construct
  REGION 1..8: note = HCDR2
INTYTGEP

SEQ ID NO: 30 - protein, 16 aa, synthetic construct
  REGION 1..16: note = HCDR3
AKYPHYYGSSHWYFDV

SEQ ID NO: 31 - protein, 6 aa, synthetic construct
  REGION 1..6: note = LCDR1
QDISNY

SEQ ID NO: 32 - skipped

SEQ ID NO: 33 - protein, 9 aa, synthetic construct
  REGION 1..9: note = LCDR3
QQYSTVPWT

SEQ ID NO: 34 - protein, 8 aa, synthetic construct
  REGION 1..8: note = HCDR1
GFAFSSYD

SEQ ID NO: 35 - protein, 8 aa, synthetic construct
  REGION 1..8: note = HCDR2
ISGGGRYT

SEQ ID NO: 36 - protein, 11 aa, synthetic construct
  REGION 1..11: note = HCDR3
ANRYGEAWFAY

SEQ ID NO: 37 - protein, 6 aa, synthetic construct
  REGION 1..6: note = LCDR1
QDINTY

SEQ ID NO: 38 - skipped

SEQ ID NO: 39 - protein, 9 aa, synthetic construct
  REGION 1..9: note = LCDR3
LQYDEFPLT

SEQ ID NO: 40 - protein, 330 aa, synthetic construct [sequence omitted]

SEQ ID NO: 41 - protein, 327 aa, synthetic construct
  REGION 1..327: note = Ig gamma-4 chain C region
ASTKGPSVFPLAPCSRSTSESTAALGCLVKDYFPEPVTVSWNSGALTSGVHTFPAVLQSSGLYSLSSVVTVPSSSLGTKTYTCNVDHKPSNTKVDKRVESKYGPPCPSCPAPEFLGGPSVFLFPPKPKDTLMISRTPEVTCVVVDVSQEDPEVQFNWYVDGVEVHNAKTKPREEQFNSTYRVVSVLTVLHQDWLNGKEYKCKVSNKGLPSSIEKTISKAKGQPREPQVYTLPPSQEEMTKNQVSLTCLVKGFYPSDIAVEWESNGQPENNYKTTPPVLDSDGSFFLYSRLTVDKSRWQEGNVFSCSVMHEALHNHYTQKSLSLSLGK

SEQ ID NO: 42 - protein, 107 aa, synthetic construct [sequence omitted]